European Patent Specification EP 3 423 075 B1, published April 3, 2024. Title: STAPLED INTRACELLULAR-TARGETING ANTIMICROBIAL PEPTIDES TO TREAT INFECTION. Applicant: DANA-FARBER CANCER INSTITUTE, INC. Application 2017-02-28. The sequence listing filed with the application follows.

SEQUENCE LISTING (60 sequences)

SEQ ID NO: 1 - protein, 25 aa, Pseudopleuronectes americanus
  C-term NH2
GWGSFFKKAAHVGKHVGKAALTHYL

SEQ ID NO: 2 - protein, 51 aa, Hippoglossus hippoglossus
SGRGKTGGKARAKAKTRSSRAGLQFPVGRVHRLLRKGNYAHRVGAGAPVYL

SEQ ID NO: 3 - protein, 39 aa, Himantura pastinacoides
KAKSRSSRAGLQFPVGRVHRLLRKGNYAERVGAGAPVYL

SEQ ID NO: 4 - protein, 51 aa, Oncorhynchus mykiss
SGRGKTGGKARAKAKTRSSRAGLQFPVGRVHRLLRKGNYAERVGAGAPVYL

SEQ ID NO: 5 - protein, 40 aa, Haliotis discus
MSGRGKGGKTKAKAKSRSSRAGLQFPVGRIHRLLRKGNYA

SEQ ID NO: 6 - protein, 40 aa, Chlamys farreri
MSGRGKGGKVKGKAKSRSSRAGLQFPVGRIHRLLRKGNYA

SEQ ID NO: 7 - protein, 21 aa, Bufo garagrizans
TRSSRAGLQFPVGRVHRLLRK

SEQ ID NO: 8 - protein, 10 aa, Homo sapiens
KLNKKAASGE

SEQ ID NO: 9 - protein, 15 aa, Homo sapiens
KLNKKAASGEAKPKA

SEQ ID NO: 10 - protein, 10 aa, Homo sapiens
KAKSPKKAKA

SEQ ID NO: 11 - protein, 24 aa, Homo sapiens
DSHAKRKKGYKRKFHEKHHSHRGY

SEQ ID NO: 12 - protein, 19 aa, Drosophila sp.
  MOD_RES (11)..(11): Glycosylated
GKPRPYSPRPTSHPRPIRV

SEQ ID NO: 13 - protein, 18 aa, Apis mellifera
GNNRPVYIPQPRPPHPRL

SEQ ID NO: 14 - protein, 25 aa, Artificial Sequence
  Description of Artificial Sequence: Synthetic peptide
  MOD_RES (3)..(3): Any amino acid whose side chain has been replaced by an internal staple
  MOD_RES (7)..(7): Any amino acid whose side chain has been replaced by an internal staple
  MOD_RES (12)..(12): Any amino acid whose side chain has been replaced by an internal staple
  MOD_RES (16)..(16): Any amino acid whose side chain has been replaced by an internal staple
  C-term NH2
GWXSFFXKAAHXGKHXGKAALTHYL

SEQ ID NO: 15 - protein, 25 aa, Artificial Sequence
  Description of Artificial Sequence: Synthetic peptide
  MOD_RES (9)..(9): Any amino acid whose side chain has been replaced by an internal staple
  MOD_RES (13)..(13): Any amino acid whose side chain has been replaced by an internal staple
  MOD_RES (19)..(19): Any amino acid whose side chain has been replaced by an internal staple
  MOD_RES (23)..(23): Any amino acid whose side chain has been replaced by an internal staple
  C-term NH2
GWGSFFKKXAHVXKHVGKXALTXYL

SEQ ID NO: 16 - protein, 51 aa, Artificial Sequence
  Description of Artificial Sequence: Synthetic polypeptide
  MOD_RES (4)..(4): Any amino acid whose side chain has been replaced by an internal staple
  MOD_RES (11)..(11): Any amino acid whose side chain has been replaced by an internal staple
SGRXKTGGKAXAKAKTRSSRAGLQFPVGRVHRLLRKGNYAHRVGAGAPVYL

SEQ ID NO: 17 - protein, 51 aa, Artificial Sequence
  Description of Artificial Sequence: Synthetic polypeptide
  MOD_RES (10)..(10): Any amino acid whose side chain has been replaced by an internal staple
  MOD_RES (14)..(14): Any amino acid whose side chain has been replaced by an internal staple
  MOD_RES (27)..(27): Any amino acid whose side chain has been replaced by an internal staple
  MOD_RES (31)..(31): Any amino acid whose side chain has been replaced by an internal staple
SGRGKTGGKXRAKXKTRSSRAGLQFPXGRVXRLLRKGNYAHRVGAGAPVYL

SEQ ID NO: 18 - protein, 39 aa, Artificial Sequence
  Description of Artificial Sequence: Synthetic polypeptide
  MOD_RES (6)..(6): Any amino acid whose side chain has been replaced by an internal staple
  MOD_RES (10)..(10): Any amino acid whose side chain has been replaced by an internal staple
  MOD_RES (29)..(29): Any amino acid whose side chain has been replaced by an internal staple
  MOD_RES (36)..(36): Any amino acid whose side chain has been replaced by an internal staple
KAKSRXSRAXLQFPVGRVHRLLRKGNYAXRVGAGAXVYL

SEQ ID NO: 19 - protein, 39 aa, Artificial Sequence
  Description of Artificial Sequence: Synthetic polypeptide
  MOD_RES (12)..(12): Any amino acid whose side chain has been replaced by an internal staple
  MOD_RES (16)..(16): Any amino acid whose side chain has been replaced by an internal staple
  MOD_RES (28)..(28): Any amino acid whose side chain has been replaced by an internal staple
  MOD_RES (35)..(35): Any amino acid whose side chain has been replaced by an internal staple
KAKSRSSRAGLXFPVXRVHRLLRKGNYXERVGAGXPVYL

SEQ ID NO: 20 - protein, 51 aa, Artificial Sequence
  Description of Artificial Sequence: Synthetic polypeptide
  MOD_RES (20)..(20): Any amino acid whose side chain has been replaced by an internal staple
  MOD_RES (27)..(27): Any amino acid whose side chain has been replaced by an internal staple
  MOD_RES (36)..(36): Any amino acid whose side chain has been replaced by an internal staple
  MOD_RES (43)..(43): Any amino acid whose side chain has been replaced by an internal staple
SGRGKTGGKARAKAKTRSSXAGLQFPXGRVHRLLRXGNYAERXGAGAPVYL

SEQ ID NO: 21 - protein, 51 aa, Artificial Sequence
  Description of Artificial Sequence: Synthetic polypeptide
  MOD_RES (10)..(10): Any amino acid whose side chain has been replaced by an internal staple
  MOD_RES (17)..(17): Any amino acid whose side chain has been replaced by an internal staple
  MOD_RES (34)..(34): Any amino acid whose side chain has been replaced by an internal staple
  MOD_RES (41)..(41): Any amino acid whose side chain has been replaced by an internal staple
SGRGKTGGKXRAKAKTXSSRAGLQFPVGRVHRLXRKGNYAXRVGAGAPVYL

SEQ ID NO: 22 - protein, 40 aa, Artificial Sequence
  Description of Artificial Sequence: Synthetic polypeptide
  MOD_RES (8)..(8): Any amino acid whose side chain has been replaced by an internal staple
  MOD_RES (15)..(15): Any amino acid whose side chain has been replaced by an internal staple
MSGRGKGXKTKAKAXSRSSRAGLQFPVGRIHRLLRKGNYA

SEQ ID NO: 23 - protein, 40 aa, Artificial Sequence
  Description of Artificial Sequence: Synthetic polypeptide
  MOD_RES (27)..(27): Any amino acid whose side chain has been replaced by an internal staple
  MOD_RES (34)..(34): Any amino acid whose side chain has been replaced by an internal staple
MSGRGKGGKTKAKAKSRSSRAGLQFPXGRIHRLXRKGNYA

SEQ ID NO: 24 - protein, 40 aa, Artificial Sequence
  Description of Artificial Sequence: Synthetic polypeptide
  MOD_RES (1)..(1): Any amino acid whose side chain has been replaced by an internal staple
  MOD_RES (8)..(8): Any amino acid whose side chain has been replaced by an internal staple
XSGRGKGXKVKGKAKSRSSRAGLQFPVGRIHRLLRKGNYA

SEQ ID NO: 25 - protein, 40 aa, Artificial Sequence
  Description of Artificial Sequence: Synthetic polypeptide
  MOD_RES (14)..(14): Any amino acid whose side chain has been replaced by an internal staple
  MOD_RES (21)..(21): Any amino acid whose side chain has been replaced by an internal staple
MSGRGKGGKVKGKXKSRSSRXGLQFPVGRIHRLLRKGNYA

SEQ ID NO: 26 - protein, 21 aa, Artificial Sequence
  Description of Artificial Sequence: Synthetic peptide
  MOD_RES (12)..(12): Any amino acid whose side chain has been replaced by an internal staple
  MOD_RES (15)..(15): Any amino acid whose side chain has been replaced by an internal staple
TRSSRAGLQFPXGRXHRLLRK

SEQ ID NO: 27 - protein, 21 aa, Artificial Sequence
  Description of Artificial Sequence: Synthetic peptide
  MOD_RES (15)..(15): Any amino acid whose side chain has been replaced by an internal staple
  MOD_RES (19)..(19): Any amino acid whose side chain has been replaced by an internal staple
TRSSRAGLQFPVGRXHRLXRK

SEQ ID NO: 28 - protein, 21 aa, Artificial Sequence
  Description of Artificial Sequence: Synthetic peptide
  MOD_RES (12)..(12): Any amino acid whose side chain has been replaced by an internal staple
  MOD_RES (19)..(19): Any amino acid whose side chain has been replaced by an internal staple
TRSSRAGLQFPXGRVHRLXRK

SEQ ID NO: 29 - protein, 15 aa, Artificial Sequence
  Description of Artificial Sequence: Synthetic peptide
  MOD_RES (2)..(2): Any amino acid whose side chain has been replaced by an internal staple
  MOD_RES (6)..(6): Any amino acid whose side chain has been replaced by an internal staple
KXNKKXASGEAKPKA

SEQ ID NO: 30 - protein, 10 aa, Artificial Sequence
  Description of Artificial Sequence: Synthetic peptide
  MOD_RES (3)..(3): Any amino acid whose side chain has been replaced by an internal staple
  MOD_RES (10)..(10): Any amino acid whose side chain has been replaced by an internal staple
KAXSPKKAKX

SEQ ID NO: 31 - protein, 24 aa, Artificial Sequence
  Description of Artificial Sequence: Synthetic peptide
  MOD_RES (5)..(5): Any amino acid whose side chain has been replaced by an internal staple
  MOD_RES (13)..(13): Any amino acid whose side chain has been replaced by an internal staple
DSHAXRKKGYKRXFHEKHHSHRGY

SEQ ID NO: 32 - protein, 24 aa, Artificial Sequence
  Description of Artificial Sequence: Synthetic peptide
  MOD_RES (3)..(3): Any amino acid whose side chain has been replaced by an internal staple
  MOD_RES (7)..(7): Any amino acid whose side chain has been replaced by an internal staple
  MOD_RES (14)..(14): Any amino acid whose side chain has been replaced by an internal staple
  MOD_RES (21)..(21): Any amino acid whose side chain has been replaced by an internal staple
DSXAKRXKGYKRKXHEKHHSXRGY

SEQ ID NO: 33 - protein, 19 aa, Artificial Sequence
  Description of Artificial Sequence: Synthetic peptide
  MOD_RES (1)..(1): Any amino acid whose side chain has been replaced by an internal staple
  MOD_RES (8)..(8): Any amino acid whose side chain has been replaced by an internal staple
  MOD_RES (11)..(11): Glycosylated
XKPRPYSXRPTSHPRPIRV

SEQ ID NO: 34 - protein, 19 aa, Artificial Sequence
  Description of Artificial Sequence: Synthetic peptide
  MOD_RES (7)..(7): Any amino acid whose side chain has been replaced by an internal staple
  MOD_RES (11)..(11): Glycosylated
  MOD_RES (14)..(14): Any amino acid whose side chain has been replaced by an internal staple
GKPRPYXPRPTSHXRPIRV

SEQ ID NO: 35 - protein, 18 aa, Artificial Sequence
  Description of Artificial Sequence: Synthetic peptide
  MOD_RES (6)..(6): Any amino acid whose side chain has been replaced by an internal staple
  MOD_RES (13)..(13): Any amino acid whose side chain has been replaced by an internal staple
GNNRPXYIPQPRXPHPRL

SEQ ID NO: 36 - protein, 18 aa, Artificial Sequence
  Description of Artificial Sequence: Synthetic peptide
  MOD_RES (4)..(4): Any amino acid whose side chain has been replaced by an internal staple
  MOD_RES (8)..(8): Any amino acid whose side chain has been replaced by an internal staple
  MOD_RES (15)..(15): Any amino acid whose side chain has been replaced by an internal staple
  MOD_RES (18)..(18): Any amino acid whose side chain has been replaced by an internal staple
GNNXPVYXPQPRPPXPRX

SEQ ID NO: 37 - protein, 21 aa, Artificial Sequence
  Description of Artificial Sequence: Synthetic peptide
  MOD_RES (17)..(17): (S)-2-(4'-pentenyl)alanine
  MOD_RES (21)..(21): (S)-2-(4'-pentenyl)alanine
TRSSRAGLQWPVGRVHALLRA

SEQ ID NO: 38 - protein, 21 aa, Artificial Sequence
  Description of Artificial Sequence: Synthetic peptide
  MOD_RES (16)..(16): (S)-2-(4'-pentenyl)alanine
  MOD_RES (20)..(20): (S)-2-(4'-pentenyl)alanine
TRSSRAGLQWPVGRVARLLAK

SEQ ID NO: 39 - protein, 21 aa, Artificial Sequence
  Description of Artificial Sequence: Synthetic peptide
  MOD_RES (15)..(15): (S)-2-(4'-pentenyl)alanine
  MOD_RES (19)..(19): (S)-2-(4'-pentenyl)alanine
TRSSRAGLQWPVGRAHRLARK

SEQ ID NO: 40 - protein, 21 aa, Artificial Sequence
  Description of Artificial Sequence: Synthetic peptide
  MOD_RES (14)..(14): (S)-2-(4'-pentenyl)alanine
  MOD_RES (18)..(18): (S)-2-(4'-pentenyl)alanine
TRSSRAGLQWPVGAVHRALRK

SEQ ID NO: 41 - protein, 21 aa, Artificial Sequence
  Description of Artificial Sequence: Synthetic peptide
  MOD_RES (13)..(13): (S)-2-(4'-pentenyl)alanine
  MOD_RES (17)..(17): (S)-2-(4'-pentenyl)alanine
TRSSRAGLQWPVARVHALLRK

SEQ ID NO: 42 - protein, 21 aa, Artificial Sequence
  Description of Artificial Sequence: Synthetic peptide
  MOD_RES (12)..(12): (S)-2-(4'-pentenyl)alanine
  MOD_RES (16)..(16): (S)-2-(4'-pentenyl)alanine
TRSSRAGLQWPAGRVARLLRK

SEQ ID NO: 43 - protein, 21 aa, Artificial Sequence
  Description of Artificial Sequence: Synthetic peptide
  MOD_RES (9)..(9): (S)-2-(4'-pentenyl)alanine
  MOD_RES (13)..(13): (S)-2-(4'-pentenyl)alanine
TRSSRAGLAWPVARVHRLLRK

SEQ ID NO: 44 - protein, 21 aa, Artificial Sequence
  Description of Artificial Sequence: Synthetic peptide
  MOD_RES (8)..(8): (S)-2-(4'-pentenyl)alanine
  MOD_RES (12)..(12): (S)-2-(4'-pentenyl)alanine
TRSSRAGAQWPAGRVHRLLRK

SEQ ID NO: 45 - protein, 21 aa, Artificial Sequence
  Description of Artificial Sequence: Synthetic peptide
  MOD_RES (5)..(5): (S)-2-(4'-pentenyl)alanine
  MOD_RES (9)..(9): (S)-2-(4'-pentenyl)alanine
TRSSAAGLAWPVGRVHRLLRK

SEQ ID NO: 46 - protein, 21 aa, Artificial Sequence
  Description of Artificial Sequence: Synthetic peptide
  MOD_RES (4)..(4): (S)-2-(4'-pentenyl)alanine
  MOD_RES (8)..(8): (S)-2-(4'-pentenyl)alanine
TRSARAGAQWPVGRVHRLLRK

SEQ ID NO: 47 - protein, 21 aa, Artificial Sequence
  Description of Artificial Sequence: Synthetic peptide
  MOD_RES (3)..(3): (S)-2-(4'-pentenyl)alanine
  MOD_RES (7)..(7): (S)-2-(4'-pentenyl)alanine
TRASRAALQWPVGRVHRLLRK

SEQ ID NO: 48 - protein, 21 aa, Artificial Sequence
  Description of Artificial Sequence: Synthetic peptide
  MOD_RES (2)..(2): (S)-2-(4'-pentenyl)alanine
  MOD_RES (6)..(6): (S)-2-(4'-pentenyl)alanine
TASSRAGLQWPVGRVHRLLRK

SEQ ID NO: 49 - protein, 21 aa, Artificial Sequence
  Description of Artificial Sequence: Synthetic peptide
  MOD_RES (1)..(1): (S)-2-(4'-pentenyl)alanine
  MOD_RES (5)..(5): (S)-2-(4'-pentenyl)alanine
ARSSAAGLQWPVGRVHRLLRK

SEQ ID NO: 50 - protein, 21 aa, Artificial Sequence
  Description of Artificial Sequence: Synthetic peptide
  MOD_RES (14)..(14): (R)-2-(7'-octenyl)alanine
  MOD_RES (21)..(21): (S)-2-(4'-pentenyl)alanine
TRSSRAGLQWPVGAVHRLLRA

SEQ ID NO: 51 - protein, 21 aa, Artificial Sequence
  Description of Artificial Sequence: Synthetic peptide
  MOD_RES (13)..(13): (R)-2-(7'-octenyl)alanine
  MOD_RES (20)..(20): (S)-2-(4'-pentenyl)alanine
TRSSRAGLQWPVARVHRLLAK

SEQ ID NO: 52 - protein, 21 aa, Artificial Sequence
  Description of Artificial Sequence: Synthetic peptide
  MOD_RES (12)..(12): (R)-2-(7'-octenyl)alanine
  MOD_RES (19)..(19): (S)-2-(4'-pentenyl)alanine
TRSSRAGLQWPAGRVHRLARK

SEQ ID NO: 53 - protein, 21 aa, Artificial Sequence
  Description of Artificial Sequence: Synthetic peptide
  MOD_RES (9)..(9): (R)-2-(7'-octenyl)alanine
  MOD_RES (16)..(16): (S)-2-(4'-pentenyl)alanine
TRSSRAGLAWPVGRVARLLRK

SEQ ID NO: 54 - protein, 21 aa, Artificial Sequence
  Description of Artificial Sequence: Synthetic peptide
  MOD_RES (8)..(8): (R)-2-(7'-octenyl)alanine
  MOD_RES (15)..(15): (S)-2-(4'-pentenyl)alanine
TRSSRAGAQWPVGRAHRLLRK

SEQ ID NO: 55 - protein, 21 aa, Artificial Sequence
  Description of Artificial Sequence: Synthetic peptide
  MOD_RES (7)..(7): (R)-2-(7'-octenyl)alanine
  MOD_RES (14)..(14): (S)-2-(4'-pentenyl)alanine
TRSSRAALQWPVGAVHRLLRK

SEQ ID NO: 56 - protein, 21 aa, Artificial Sequence
  Description of Artificial Sequence: Synthetic peptide
  MOD_RES (6)..(6): (R)-2-(7'-octenyl)alanine
  MOD_RES (13)..(13): (S)-2-(4'-pentenyl)alanine
TRSSRAGLQWPVARVHRLLRK

SEQ ID NO: 57 - protein, 21 aa, Artificial Sequence
  Description of Artificial Sequence: Synthetic peptide
  MOD_RES (5)..(5): (R)-2-(7'-octenyl)alanine
  MOD_RES (12)..(12): (S)-2-(4'-pentenyl)alanine
TRSSAAGLQWPAGRVHRLLRK

SEQ ID NO: 58 - protein, 21 aa, Artificial Sequence
  Description of Artificial Sequence: Synthetic peptide
  MOD_RES (2)..(2): (R)-2-(7'-octenyl)alanine
  MOD_RES (9)..(9): (S)-2-(4'-pentenyl)alanine
TASSRAGLAWPVGRVHRLLRK

SEQ ID NO: 59 - protein, 21 aa, Artificial Sequence
  Description of Artificial Sequence: Synthetic peptide
  MOD_RES (1)..(1): (R)-2-(7'-octenyl)alanine
  MOD_RES (8)..(8): (S)-2-(4'-pentenyl)alanine
ARSSRAGAQWPVGRVHRLLRK

SEQ ID NO: 60 - protein, 21 aa, Artificial Sequence
  Description of Artificial Sequence: Synthetic peptide
TRSSRAGLQWPVGRVHRLLRK